European Patent Specification EP 3 245 215 B9, published October 4, 2023. Title: METHODS OF TREATING NEUROLOGICAL INFLAMMATORY DISORDERS. Applicant: Mayo Foundation for Medical Education and Research. The sequence listing filed with the application follows.

SEQUENCE LISTING (144 sequences)

SEQ ID NO: 1 - DNA, 23 bp, Artificial Sequence
  synthetic oligonucleotide
tggtctcatcagttattcccatc

SEQ ID NO: 2 - DNA, 21 bp, Artificial Sequence
  synthetic oligonucleotide
cgagaaatgatggagtctgga

SEQ ID NO: 3 - DNA, 21 bp, Artificial Sequence
  synthetic oligonucleotide
tgatcttcatgctcagatcca

SEQ ID NO: 4 - DNA, 19 bp, Artificial Sequence
  synthetic oligonucleotide
gcaaatgttgttggcaagc

SEQ ID NO: 5 - DNA, 22 bp, Artificial Sequence
  synthetic oligonucleotide
tgaataaaaaggcaacctaccg

SEQ ID NO: 6 - DNA, 22 bp, Artificial Sequence
  synthetic oligonucleotide
tgggagatgtcaatctctgttc

SEQ ID NO: 7 - DNA, 25 bp, Artificial Sequence
  synthetic oligonucleotide
tgagaaaagcttctaaacagaaagg

SEQ ID NO: 8 - DNA, 20 bp, Artificial Sequence
  synthetic oligonucleotide
gtactggccctggtttaacg

SEQ ID NO: 9 - DNA, 21 bp, Artificial Sequence
  synthetic oligonucleotide
aagcaaagtccacacttccag

SEQ ID NO: 10 - DNA, 20 bp, Artificial Sequence
  synthetic oligonucleotide
gtagtaccgggaggctgacc

SEQ ID NO: 11 - DNA, 19 bp, Artificial Sequence
  synthetic oligonucleotide
ggatgtggtggacatcgtg

SEQ ID NO: 12 - DNA, 18 bp, Artificial Sequence
  synthetic oligonucleotide
gaggccgatggttctcag

SEQ ID NO: 13 - DNA, 20 bp, Artificial Sequence
  synthetic oligonucleotide
tattccatcggcttggtttg

SEQ ID NO: 14 - DNA, 20 bp, Artificial Sequence
  synthetic oligonucleotide
tgtgagctgaagacacagca

SEQ ID NO: 15 - DNA, 19 bp, Artificial Sequence
  synthetic oligonucleotide
ggccagatgaccgtctacc

SEQ ID NO: 16 - DNA, 18 bp, Artificial Sequence
  synthetic oligonucleotide
gccgtctgcacagttggt

SEQ ID NO: 17 - DNA, 20 bp, Artificial Sequence
  synthetic oligonucleotide
tctaccatgagcatcggtgt

SEQ ID NO: 18 - DNA, 21 bp, Artificial Sequence
  synthetic oligonucleotide
catcgaagacctcagagccta

SEQ ID NO: 19 - DNA, 18 bp, Artificial Sequence
  synthetic oligonucleotide
agggattccggacctttg

SEQ ID NO: 20 - DNA, 20 bp, Artificial Sequence
  synthetic oligonucleotide
gcagcagtttgggttgtttc

SEQ ID NO: 21 - DNA, 20 bp, Artificial Sequence
  synthetic oligonucleotide
gccatcactgtgtcatctgc

SEQ ID NO: 22 - DNA, 20 bp, Artificial Sequence
  synthetic oligonucleotide
catcttgaatccaccgaagg

SEQ ID NO: 23 - DNA, 19 bp, Artificial Sequence
  synthetic oligonucleotide
catggtatcctccgcaatg

SEQ ID NO: 24 - DNA, 21 bp, Artificial Sequence
  synthetic oligonucleotide
gcgcatttaaggcattgtaac

SEQ ID NO: 25 - DNA, 21 bp, Artificial Sequence
  synthetic oligonucleotide
aacctggacaaagcactgaag

SEQ ID NO: 26 - DNA, 22 bp, Artificial Sequence
  synthetic oligonucleotide
aatgcattgtagcagttgatcc

SEQ ID NO: 27 - DNA, 21 bp, Artificial Sequence
  synthetic oligonucleotide
caagctggctgacttaatgga

SEQ ID NO: 28 - DNA, 20 bp, Artificial Sequence
  synthetic oligonucleotide
gactttcccagcattcatcg

SEQ ID NO: 29 - DNA, 21 bp, Artificial Sequence
  synthetic oligonucleotide
gaccggagaacgctgatacta

SEQ ID NO: 30 - DNA, 18 bp, Artificial Sequence
  synthetic oligonucleotide
agtcgggcagtcagcatc

SEQ ID NO: 31 - DNA, 20 bp, Artificial Sequence
  synthetic oligonucleotide
tccctacttcccgtctttga

SEQ ID NO: 32 - DNA, 19 bp, Artificial Sequence
  synthetic oligonucleotide
acaggctctgcccgattac

SEQ ID NO: 33 - DNA, 20 bp, Artificial Sequence
  synthetic oligonucleotide
cgctcgctcctctacatcat

SEQ ID NO: 34 - DNA, 21 bp, Artificial Sequence
  synthetic oligonucleotide
gccaacttcagcttgtttttg

SEQ ID NO: 35 - DNA, 20 bp, Artificial Sequence
  synthetic oligonucleotide
tgttcggggacgtaaaagac

SEQ ID NO: 36 - DNA, 20 bp, Artificial Sequence
  synthetic oligonucleotide
tgaggatttgcatcactggt

SEQ ID NO: 37 - DNA, 23 bp, Artificial Sequence
  synthetic oligonucleotide
tgtggagaagctcaaaaagtcac

SEQ ID NO: 38 - DNA, 20 bp, Artificial Sequence
  synthetic oligonucleotide
cccatagtcatgggactgct

SEQ ID NO: 39 - DNA, 21 bp, Artificial Sequence
  synthetic oligonucleotide
gctgaagcagttcaacaaagg

SEQ ID NO: 40 - DNA, 21 bp, Artificial Sequence
  synthetic oligonucleotide
aggagaggcaacaaggaagtc

SEQ ID NO: 41 - DNA, 20 bp, Artificial Sequence
  synthetic oligonucleotide
ctggatgaagccatcgagtt

SEQ ID NO: 42 - DNA, 22 bp, Artificial Sequence
  synthetic oligonucleotide
ccaacacctgtttgataacctg

SEQ ID NO: 43 - DNA, 20 bp, Artificial Sequence
  synthetic oligonucleotide
aagagttgctgcacatctgg

SEQ ID NO: 44 - DNA, 18 bp, Artificial Sequence
  synthetic oligonucleotide
gtgcagtgtggcctcaga

SEQ ID NO: 45 - DNA, 18 bp, Artificial Sequence
  synthetic oligonucleotide
accggttccgtaccttcc

SEQ ID NO: 46 - DNA, 21 bp, Artificial Sequence
  synthetic oligonucleotide
agctgtgcacaaaatggaaat

SEQ ID NO: 47 - DNA, 20 bp, Artificial Sequence
  synthetic oligonucleotide
aacagctggaaaggggtctc

SEQ ID NO: 48 - DNA, 25 bp, Artificial Sequence
  synthetic oligonucleotide
cattaagtcgtaccatttacggagt

SEQ ID NO: 49 - DNA, 21 bp, Artificial Sequence
  synthetic oligonucleotide
ggtaaatgccacatggtatcc

SEQ ID NO: 50 - DNA, 24 bp, Artificial Sequence
  synthetic oligonucleotide
tgattcaacaaattttccatcaat

SEQ ID NO: 51 - DNA, 20 bp, Artificial Sequence
  synthetic oligonucleotide
tgtccttcactgggagcact

SEQ ID NO: 52 - DNA, 20 bp, Artificial Sequence
  synthetic oligonucleotide
gtttcctccaagctccaaca

SEQ ID NO: 53 - DNA, 22 bp, Artificial Sequence
  synthetic oligonucleotide
ggcaagaatcctgctatcatct

SEQ ID NO: 54 - DNA, 22 bp, Artificial Sequence
  synthetic oligonucleotide
actggtacaaaggcaaatctcc

SEQ ID NO: 55 - DNA, 20 bp, Artificial Sequence
  synthetic oligonucleotide
ctggcagtgcctggaatact

SEQ ID NO: 56 - DNA, 19 bp, Artificial Sequence
  synthetic oligonucleotide
cctcctgggagctgaatgt

SEQ ID NO: 57 - DNA, 18 bp, Artificial Sequence
  synthetic oligonucleotide
ctcttgggccaccatgtc

SEQ ID NO: 58 - DNA, 19 bp, Artificial Sequence
  synthetic oligonucleotide
ctggccaggttttctcctg

SEQ ID NO: 59 - DNA, 22 bp, Artificial Sequence
  synthetic oligonucleotide
gatgtcatcgtcacagagaacg

SEQ ID NO: 60 - DNA, 18 bp, Artificial Sequence
  synthetic oligonucleotide
aagacacaggcgctgtcc

SEQ ID NO: 61 - DNA, 19 bp, Artificial Sequence
  synthetic oligonucleotide
gcctcaccaaacagattgc

SEQ ID NO: 62 - DNA, 18 bp, Artificial Sequence
  synthetic oligonucleotide
cacgcctcgcattaccat

SEQ ID NO: 63 - DNA, 20 bp, Artificial Sequence
  synthetic oligonucleotide
ggcgttcgtgattactgtga

SEQ ID NO: 64 - DNA, 21 bp, Artificial Sequence
  synthetic oligonucleotide
tcttcctcatgtccaaatcca

SEQ ID NO: 65 - DNA, 18 bp, Artificial Sequence
  synthetic oligonucleotide
ctttgccacggacgagac

SEQ ID NO: 66 - DNA, 22 bp, Artificial Sequence
  synthetic oligonucleotide
tcattgtactctgagggctgac

SEQ ID NO: 67 - DNA, 20 bp, Artificial Sequence
  synthetic oligonucleotide
caacacaaggaactgcttcg

SEQ ID NO: 68 - DNA, 20 bp, Artificial Sequence
  synthetic oligonucleotide
gatttagcatggggctcttg

SEQ ID NO: 69 - DNA, 21 bp, Artificial Sequence
  synthetic oligonucleotide
cataaggagttccttcgtctc

SEQ ID NO: 70 - DNA, 25 bp, Artificial Sequence
  synthetic oligonucleotide
cgactttcacgagtaacatcttctt

SEQ ID NO: 71 - DNA, 19 bp, Artificial Sequence
  synthetic oligonucleotide
gggaagccgcactgttact

SEQ ID NO: 72 - DNA, 19 bp, Artificial Sequence
  synthetic oligonucleotide
gagatcgcgcactgtttgt

SEQ ID NO: 73 - DNA, 20 bp, Artificial Sequence
  synthetic oligonucleotide
ctgatgctagtgctgccaga

SEQ ID NO: 74 - DNA, 20 bp, Artificial Sequence
  synthetic oligonucleotide
gtgcactctgaggccaaact

SEQ ID NO: 75 - DNA, 20 bp, Artificial Sequence
  synthetic oligonucleotide
gcccactaaaattcggaagc

SEQ ID NO: 76 - DNA, 22 bp, Artificial Sequence
  synthetic oligonucleotide
cttctgctacaaccactgaacg

SEQ ID NO: 77 - DNA, 20 bp, Artificial Sequence
  synthetic oligonucleotide
acaaaaagaggatgggcttg

SEQ ID NO: 78 - DNA, 20 bp, Artificial Sequence
  synthetic oligonucleotide
tcatgacggagcctttctct

SEQ ID NO: 79 - DNA, 20 bp, Artificial Sequence
  synthetic oligonucleotide
cttgggaaggcaagaaggta

SEQ ID NO: 80 - DNA, 20 bp, Artificial Sequence
  synthetic oligonucleotide
tggagctgctggtgttttct

SEQ ID NO: 81 - DNA, 19 bp, Artificial Sequence
  synthetic oligonucleotide
aaagcctcccccagaagtt

SEQ ID NO: 82 - DNA, 21 bp, Artificial Sequence
  synthetic oligonucleotide
catgttcaaattggcatgtgt

SEQ ID NO: 83 - DNA, 27 bp, Artificial Sequence
  synthetic oligonucleotide
caagtgtctttctggattaataaggag

SEQ ID NO: 84 - DNA, 24 bp, Artificial Sequence
  synthetic oligonucleotide
gtcatggttaaaacagtggtgatt

SEQ ID NO: 85 - DNA, 20 bp, Artificial Sequence
  synthetic oligonucleotide
ccctctggatgagcaaaact

SEQ ID NO: 86 - DNA, 21 bp, Artificial Sequence
  synthetic oligonucleotide
aattcgatgtcatccgtggta

SEQ ID NO: 87 - DNA, 25 bp, Artificial Sequence
  synthetic oligonucleotide
gggtctccttttggattaactatga

SEQ ID NO: 88 - DNA, 26 bp, Artificial Sequence
  synthetic oligonucleotide
ggtcattgttaggacagttgtaattc

SEQ ID NO: 89 - DNA, 21 bp, Artificial Sequence
  synthetic oligonucleotide
ctccattgtagagcaccgtct

SEQ ID NO: 90 - DNA, 22 bp, Artificial Sequence
  synthetic oligonucleotide
tcaatgaaagtcgaggataggc

SEQ ID NO: 91 - DNA, 21 bp, Artificial Sequence
  synthetic oligonucleotide
cggagctgatgaacttcaaat

SEQ ID NO: 92 - DNA, 18 bp, Artificial Sequence
  synthetic oligonucleotide
atgtagacgccccggttc

SEQ ID NO: 93 - DNA, 20 bp, Artificial Sequence
  synthetic oligonucleotide
acagaaaatgacgctgtgga

SEQ ID NO: 94 - DNA, 22 bp, Artificial Sequence
  synthetic oligonucleotide
catctgacttttggcttgtgaa

SEQ ID NO: 95 - DNA, 19 bp, Artificial Sequence
  synthetic oligonucleotide
atgcgacaccagcaagaac

SEQ ID NO: 96 - DNA, 20 bp, Artificial Sequence
  synthetic oligonucleotide
caatggtgctgagtgtggtc

SEQ ID NO: 97 - DNA, 20 bp, Artificial Sequence
  synthetic oligonucleotide
atttcaccctggtcaccgta

SEQ ID NO: 98 - DNA, 21 bp, Artificial Sequence
  synthetic oligonucleotide
gctcaaattgcaaaaccaatc

SEQ ID NO: 99 - DNA, 20 bp, Artificial Sequence
  synthetic oligonucleotide
tgcctgctagagtcccctta

SEQ ID NO: 100 - DNA, 19 bp, Artificial Sequence
  synthetic oligonucleotide
ccgtgatgatggtggacat

SEQ ID NO: 101 - DNA, 22 bp, Artificial Sequence
  synthetic oligonucleotide
gacattgatgtctccattctgc

SEQ ID NO: 102 - DNA, 21 bp, Artificial Sequence
  synthetic oligonucleotide
gcagccctttgtaaccataga

SEQ ID NO: 103 - DNA, 20 bp, Artificial Sequence
  synthetic oligonucleotide
gaacatggcagcgaaagtct

SEQ ID NO: 104 - DNA, 20 bp, Artificial Sequence
  synthetic oligonucleotide
ctggtacttgctgccaaaca

SEQ ID NO: 105 - DNA, 20 bp, Artificial Sequence
  synthetic oligonucleotide
agggatcgacatccagagag

SEQ ID NO: 106 - DNA, 20 bp, Artificial Sequence
  synthetic oligonucleotide
tgcacatttcctgtcaaacc

SEQ ID NO: 107 - DNA, 18 bp, Artificial Sequence
  synthetic oligonucleotide
ggggaggtgattccaagg

SEQ ID NO: 108 - DNA, 19 bp, Artificial Sequence
  synthetic oligonucleotide
cccccgacaaggatgtaga

SEQ ID NO: 109 - DNA, 20 bp, Artificial Sequence
  synthetic oligonucleotide
agccgtgtgatacgatgaaa

SEQ ID NO: 110 - DNA, 20 bp, Artificial Sequence
  synthetic oligonucleotide
caaggtttacaggcgttcct

SEQ ID NO: 111 - DNA, 20 bp, Artificial Sequence
  synthetic oligonucleotide
ctgccaacagttttgctgtg

SEQ ID NO: 112 - DNA, 20 bp, Artificial Sequence
  synthetic oligonucleotide
aaatggcaaacacccctcta

SEQ ID NO: 113 - DNA, 21 bp, Artificial Sequence
  synthetic oligonucleotide
agacttttggcaaagacatgc

SEQ ID NO: 114 - DNA, 19 bp, Artificial Sequence
  synthetic oligonucleotide
actgccattcaagcccttc

SEQ ID NO: 115 - DNA, 21 bp, Artificial Sequence
  synthetic oligonucleotide
ccctaccgtgatgtcttttca

SEQ ID NO: 116 - DNA, 20 bp, Artificial Sequence
  synthetic oligonucleotide
agaatgtccatgtcgccact

SEQ ID NO: 117 - DNA, 18 bp, Artificial Sequence
  synthetic oligonucleotide
tctggtttggcgttggag

SEQ ID NO: 118 - DNA, 22 bp, Artificial Sequence
  synthetic oligonucleotide
tcctccaactattctggtcgat

SEQ ID NO: 119 - DNA, 20 bp, Artificial Sequence
  synthetic oligonucleotide
agtgccaccataccatccag

SEQ ID NO: 120 - DNA, 21 bp, Artificial Sequence
  synthetic oligonucleotide
gctggcacttcagagacattc

SEQ ID NO: 121 - DNA, 22 bp, Artificial Sequence
  synthetic oligonucleotide
cacttcatcttcaccactctgg

SEQ ID NO: 122 - DNA, 19 bp, Artificial Sequence
  synthetic oligonucleotide
actcccgagtagcggtagg

SEQ ID NO: 123 - DNA, 20 bp, Artificial Sequence
  synthetic oligonucleotide
gccattgagtatggcacgat

SEQ ID NO: 124 - DNA, 20 bp, Artificial Sequence
  synthetic oligonucleotide
tggtaacgggaattttggaa

SEQ ID NO: 125 - DNA, 20 bp, Artificial Sequence
  synthetic oligonucleotide
cccctcagctagcctcatct

SEQ ID NO: 126 - DNA, 20 bp, Artificial Sequence
  synthetic oligonucleotide
gcctcgcaccagttcttcta

SEQ ID NO: 127 - DNA, 21 bp, Artificial Sequence
  synthetic oligonucleotide
catttagggctatcacctcca

SEQ ID NO: 128 - DNA, 22 bp, Artificial Sequence
  synthetic oligonucleotide
cactgtgtctttttggttttgc

SEQ ID NO: 129 - DNA, 19 bp, Artificial Sequence
  synthetic oligonucleotide
attcaaccagaggggcgta

SEQ ID NO: 130 - DNA, 21 bp, Artificial Sequence
  synthetic oligonucleotide
ttcaagacagctgcgtcatag

SEQ ID NO: 131 - DNA, 19 bp, Artificial Sequence
  synthetic oligonucleotide
gggttacaaccggtgccta

SEQ ID NO: 132 - DNA, 20 bp, Artificial Sequence
  synthetic oligonucleotide
ctttgccgatggtgaaagat

SEQ ID NO: 133 - DNA, 18 bp, Artificial Sequence
  synthetic oligonucleotide
gaagcgggccatagacct

SEQ ID NO: 134 - DNA, 18 bp, Artificial Sequence
  synthetic oligonucleotide
tggcagatccctgagagc

SEQ ID NO: 135 - DNA, 19 bp, Artificial Sequence
  synthetic oligonucleotide
tgcgatacaaccagccaag

SEQ ID NO: 136 - DNA, 20 bp, Artificial Sequence
  synthetic oligonucleotide
agatgaaggcgtccagtttc

SEQ ID NO: 137 - DNA, 22 bp, Artificial Sequence
  synthetic oligonucleotide
cacgaatcaaaaacaaatccaa

SEQ ID NO: 138 - DNA, 23 bp, Artificial Sequence
  synthetic oligonucleotide
tgtgtttaatgctctgtgaaacc

SEQ ID NO: 139 - DNA, 18 bp, Artificial Sequence
  synthetic oligonucleotide
cgtcctacggagggaggt

SEQ ID NO: 140 - DNA, 18 bp, Artificial Sequence
  synthetic oligonucleotide
ccagggacaccagcacat

SEQ ID NO: 141 - DNA, 20 bp, Artificial Sequence
  synthetic oligonucleotide
ctcaaggaggctacccacag

SEQ ID NO: 142 - DNA, 20 bp, Artificial Sequence
  synthetic oligonucleotide
tagttcccatgctgaggtga

SEQ ID NO: 143 - DNA, 20 bp, Artificial Sequence
  synthetic oligonucleotide
tctgtgcgagaggtagcaga

SEQ ID NO: 144 - DNA, 19 bp, Artificial Sequence
  synthetic oligonucleotide
cggatgaagatggcgatag